European Patent Application EP 4 365 205 A1, published May 8, 2024. Title: TRISPECIFIC ANTIBODY AND PREPARATION METHOD THEREFOR AND USE THEREOF. Applicant: SUNSHINE GUOJIAN PHARMACEUTICAL (SHANGHAI) CO., LTD. The sequence listing filed with the application follows.

SEQUENCE LISTING (19 sequences)

SEQ ID NO: 1 - protein, 117 aa, Artificial Sequence
  609-IgG4 heavy chain variable region amino acid sequence
EVKLVESGGGLVQPGGSLRLSCAASGFAFSSYDMSWVRQAPGKRLEWVATISGGGRYTYYPDTVKGRFTISRDNAKNSHYLQMNSLRAEDTAVYFCASPYGGYFDVWGQGTLVTVSS

SEQ ID NO: 2 - protein, 107 aa, Artificial Sequence
  609-IgG4 light chain variable region amino acid sequence
EIVLTQSPATLSLSPGERATLSCRASQSISNFLHWYQQKPGQAPRLLIKYASQSISGIPARFSGSGSGTDFTLTISSLEPEDFAVYFCQQSNSWPHTFGQGTKVEIK

SEQ ID NO: 3 - protein, 327 aa, Artificial Sequence
  609-IgG4 heavy chain constant region amino acid sequence
ASTKGPSVFPLAPCSRSTSESTAALGCLVKDYFPEPVTVSWNSGALTSGVHTFPAVLQSSGLYSLSSVVTVPSSSLGTKTYTCNVDHKPSNTKVDKRVESKYGPPCPPCPAPEFLGGPSVFLFPPKPKDTLMISRTPEVTCVVVDVSQEDPEVQFNWYVDGVEVHNAKTKPREEQFNSTYRVVSVLTVLHQDWLNGKEYKCKVSNKGLPSSIEKTISKAKGQPREPQVYTLPPSQEEMTKNQVSLTCLVKGFYPSDIAVEWESNGQPENNYKTTPPVLDSDGSFFLYSRLTVDKSRWQEGNVFSCSVMHEALHNHYTQKSLSLSLGK

SEQ ID NO: 4 - protein, 107 aa, Artificial Sequence [sequence omitted]

SEQ ID NO: 5 - protein, 444 aa, Artificial Sequence
  609-IgG4 heavy chain amino acid sequence
EVKLVESGGGLVQPGGSLRLSCAASGFAFSSYDMSWVRQAPGKRLEWVATISGGGRYTYYPDTVKGRFTISRDNAKNSHYLQMNSLRAEDTAVYFCASPYGGYFDVWGQGTLVTVSSASTKGPSVFPLAPCSRSTSESTAALGCLVKDYFPEPVTVSWNSGALTSGVHTFPAVLQSSGLYSLSSVVTVPSSSLGTKTYTCNVDHKPSNTKVDKRVESKYGPPCPPCPAPEFLGGPSVFLFPPKPKDTLMISRTPEVTCVVVDVSQEDPEVQFNWYVDGVEVHNAKTKPREEQFNSTYRVVSVLTVLHQDWLNGKEYKCKVSNKGLPSSIEKTISKAKGQPREPQVYTLPPSQEEMTKNQVSLTCLVKGFYPSDIAVEWESNGQPENNYKTTPPVLDSDGSFFLYSRLTVDKSRWQEGNVFSCSVMHEALHNHYTQKSLSLSLGK

SEQ ID NO: 6 - protein, 214 aa, Artificial Sequence
  609-IgG4 light chain amino acid sequence
EIVLTQSPATLSLSPGERATLSCRASQSISNFLHWYQQKPGQAPRLLIKYASQSISGIPARFSGSGSGTDFTLTISSLEPEDFAVYFCQQSNSWPHTFGQGTKVEIKRTVAAPSVFIFPPSDEQLKSGTASVVCLLNNFYPREAKVQWKVDNALQSGNSQESVTEQDSKDSTYSLSSTLTLSKADYEKHKVYACEVTHQGLSSPVTKSFNRGEC

SEQ ID NO: 7 - protein, 120 aa, Artificial Sequence [sequence omitted]

SEQ ID NO: 8 - protein, 107 aa, Artificial Sequence [sequence omitted]

SEQ ID NO: 9 - protein, 330 aa, Artificial Sequence
  Human IgG1 heavy chain constant region amino acid sequence
ASTKGPSVFPLAPSSKSTSGGTAALGCLVKDYFPEPVTVSWNSGALTSGVHTFPAVLQSSGLYSLSSVVTVPSSSLGTQTYICNVNHKPSNTKVDKKVEPKSCDKTHTCPPCPAPELLGGPSVFLFPPKPKDTLMISRTPEVTCVVVDVSHEDPEVKFNWYVDGVEVHNAKTKPREEQYNSTYRVVSVLTVLHQDWLNGKEYKCKVSNKALPAPIEKTISKAKGQPREPQVYTLPPSREEMTKNQVSLTCLVKGFYPSDIAVEWESNGQPENNYKTTPPVLDSDGSFFLYSKLTVDKSRWQQGNVFSCSVMHEALHNHYTQKSLSLSPGK

SEQ ID NO: 10 - protein, 450 aa, Artificial Sequence
  302-IgG1 heavy chain amino acid sequence
EVQLVESGGGLVQPGGSLRLSCAASGFNIKDTYIHWVRQAPGKGLEWVARIYPTNGYTRYADSVKGRFTISADTSKNTAYLQMNSLRAEDTAVYYCSRWGGDGFYAMDYWGQGTLVTVSSASTKGPSVFPLAPSSKSTSGGTAALGCLVKDYFPEPVTVSWNSGALTSGVHTFPAVLQSSGLYSLSSVVTVPSSSLGTQTYICNVNHKPSNTKVDKKVEPKSCDKTHTCPPCPAPELLGGPSVFLFPPKPKDTLMISRTPEVTCVVVDVSHEDPEVKFNWYVDGVEVHNAKTKPREEQYNSTYRVVSVLTVLHQDWLNGKEYKCKVSNKALPAPIEKTISKAKGQPREPQVYTLPPSREEMTKNQVSLTCLVKGFYPSDIAVEWESNGQPENNYKTTPPVLDSDGSFFLYSKLTVDKSRWQQGNVFSCSVMHEALHNHYTQKSLSLSPGK

SEQ ID NO: 11 - protein, 214 aa, Artificial Sequence
  302-IgG1 light chain amino acid sequence
DIQMTQSPSSLSASVGDRVTITCRASQDVNTAVAWYQQKPGKAPKLLIYSASFLYSGVPSRFSGSRSGTDFTLTISSLQPEDFATYYCQQHYTTPPTFGQGTKVEIKRTVAAPSVFIFPPSDEQLKSGTASVVCLLNNFYPREAKVQWKVDNALQSGNSQESVTEQDSKDSTYSLSSTLTLSKADYEKHKVYACEVTHQGLSSPVTKSFNRGEC

SEQ ID NO: 12 - protein, 447 aa, Artificial Sequence
  134-IgG4 heavy chain amino acid sequence
QVQLVQSGAEVKKPGASVKVSCKASGYTLTAYYMNWVRQAPGQSLEWIGVINPYNGDSSYNQKFKGRATLTVDKSTSTAYMELSSLRSEDTAVYYCARDDGYYRWYFDVWGQGTLVTVSSASTKGPSVFPLAPCSRSTSESTAALGCLVKDYFPEPVTVSWNSGALTSGVHTFPAVLQSSGLYSLSSVVTVPSSSLGTKTYTCNVDHKPSNTKVDKRVESKYGPPCPPCPAPEFLGGPSVFLFPPKPKDTLMISRTPEVTCVVVDVSQEDPEVQFNWYVDGVEVHNAKTKPREEQFNSTYRVVSVLTVLHQDWLNGKEYKCKVSNKGLPSSIEKTISKAKGQPREPQVYTLPPSQEEMTKNQVSLTCLVKGFYPSDIAVEWESNGQPENNYKTTPPVLDSDGSFFLYSRLTVDKSRWQEGNVFSCSVMHEALHNHYTQKSLSLSLGK

SEQ ID NO: 13 - protein, 214 aa, Artificial Sequence
  134-IgG4 light chain amino acid sequence
DIQMTQSPSSLSASVGDRVTITCRASQDIGSRLNWLQQKPGKSIKRLIYATSSLESGVPSRFSGSRSGSDYTLTISSLQPEDFATYYCLQSGSSPPTFGQGTKVEIKRTVAAPSVFIFPPSDEQLKSGTASVVCLLNNFYPREAKVQWKVDNALQSGNSQESVTEQDSKDSTYSLSSTLTLSKADYEKHKVYACEVTHQGLSSPVTKSFNRGEC

SEQ ID NO: 14 - protein, 714 aa, Artificial Sequence
  609VH-302VH-134-IgG4 amino acid sequence
EVKLVESGGGLVQPGGSLRLSCAASGFAFSSYDMSWVRQAPGKRLEWVATISGGGRYTYYPDTVKGRFTISRDNAKNSHYLQMNSLRAEDTAVYFCASPYGGYFDVWGQGTLVTVSSGGGGSGGGGSGGGGSEVQLVESGGGLVQPGGSLRLSCAASGFNIKDTYIHWVRQAPGKGLEWVARIYPTNGYTRYADSVKGRFTISADTSKNTAYLQMNSLRAEDTAVYYCSRWGGDGFYAMDYWGQGTLVTVSSGGGGSGGGGSGGGGSQVQLVQSGAEVKKPGASVKVSCKASGYTLTAYYMNWVRQAPGQSLEWIGVINPYNGDSSYNQKFKGRATLTVDKSTSTAYMELSSLRSEDTAVYYCARDDGYYRWYFDVWGQGTLVTVSSASTKGPSVFPLAPCSRSTSESTAALGCLVKDYFPEPVTVSWNSGALTSGVHTFPAVLQSSGLYSLSSVVTVPSSSLGTKTYTCNVDHKPSNTKVDKRVESKYGPPCPPCPAPEFLGGPSVFLFPPKPKDTLMISRTPEVTCVVVDVSQEDPEVQFNWYVDGVEVHNAKTKPREEQFNSTYRVVSVLTVLHQDWLNGKEYKCKVSNKGLPSSIEKTISKAKGQPREPQVYTLPPSQEEMTKNQVSLTCLVKGFYPSDIAVEWESNGQPENNYKTTPPVLDSDGSFFLYSRLTVDKSRWQEGNVFSCSVMHEALHNHYTQKSLSLSLGK

SEQ ID NO: 15 - protein, 229 aa, Artificial Sequence
  609VL-302VL amino acid sequence
EIVLTQSPATLSLSPGERATLSCRASQSISNFLHWYQQKPGQAPRLLIKYASQSISGIPARFSGSGSGTDFTLTISSLEPEDFAVYFCQQSNSWPHTFGQGTKVEIKGGGGSGGGGSGGGGSDIQMTQSPSSLSASVGDRVTITCRASQDVNTAVAWYQQKPGKAPKLLIYSASFLYSGVPSRFSGSRSGTDFTLTISSLQPEDFATYYCQQHYTTPPTFGQGTKVEIK

SEQ ID NO: 16 - protein, 714 aa, Artificial Sequence
  609VH-302VH(44C)-134-IgG4 amino acid sequence
EVKLVESGGGLVQPGGSLRLSCAASGFAFSSYDMSWVRQAPGKRLEWVATISGGGRYTYYPDTVKGRFTISRDNAKNSHYLQMNSLRAEDTAVYFCASPYGGYFDVWGQGTLVTVSSGGGGSGGGGSGGGGSEVQLVESGGGLVQPGGSLRLSCAASGFNIKDTYIHWVRQAPGKCLEWVARIYPTNGYTRYADSVKGRFTISADTSKNTAYLQMNSLRAEDTAVYYCSRWGGDGFYAMDYWGQGTLVTVSSGGGGSGGGGSGGGGSQVQLVQSGAEVKKPGASVKVSCKASGYTLTAYYMNWVRQAPGQSLEWIGVINPYNGDSSYNQKFKGRATLTVDKSTSTAYMELSSLRSEDTAVYYCARDDGYYRWYFDVWGQGTLVTVSSASTKGPSVFPLAPCSRSTSESTAALGCLVKDYFPEPVTVSWNSGALTSGVHTFPAVLQSSGLYSLSSVVTVPSSSLGTKTYTCNVDHKPSNTKVDKRVESKYGPPCPPCPAPEFLGGPSVFLFPPKPKDTLMISRTPEVTCVVVDVSQEDPEVQFNWYVDGVEVHNAKTKPREEQFNSTYRVVSVLTVLHQDWLNGKEYKCKVSNKGLPSSIEKTISKAKGQPREPQVYTLPPSQEEMTKNQVSLTCLVKGFYPSDIAVEWESNGQPENNYKTTPPVLDSDGSFFLYSRLTVDKSRWQEGNVFSCSVMHEALHNHYTQKSLSLSLGK

SEQ ID NO: 17 - protein, 229 aa, Artificial Sequence
  609VL-302VL(100C) amino acid sequence
EIVLTQSPATLSLSPGERATLSCRASQSISNFLHWYQQKPGQAPRLLIKYASQSISGIPARFSGSGSGTDFTLTISSLEPEDFAVYFCQQSNSWPHTFGQGTKVEIKGGGGSGGGGSGGGGSDIQMTQSPSSLSASVGDRVTITCRASQDVNTAVAWYQQKPGKAPKLLIYSASFLYSGVPSRFSGSRSGTDFTLTISSLQPEDFATYYCQQHYTTPPTFGCGTKVEIK

SEQ ID NO: 18 - protein, 714 aa, Artificial Sequence
  609VH-302VH(105C)-134-IgG4 amino acid sequence
EVKLVESGGGLVQPGGSLRLSCAASGFAFSSYDMSWVRQAPGKRLEWVATISGGGRYTYYPDTVKGRFTISRDNAKNSHYLQMNSLRAEDTAVYFCASPYGGYFDVWGQGTLVTVSSGGGGSGGGGSGGGGSEVQLVESGGGLVQPGGSLRLSCAASGFNIKDTYIHWVRQAPGKGLEWVARIYPTNGYTRYADSVKGRFTISADTSKNTAYLQMNSLRAEDTAVYYCSRWGGDGFYAMDYWGCGTLVTVSSGGGGSGGGGSGGGGSQVQLVQSGAEVKKPGASVKVSCKASGYTLTAYYMNWVRQAPGQSLEWIGVINPYNGDSSYNQKFKGRATLTVDKSTSTAYMELSSLRSEDTAVYYCARDDGYYRWYFDVWGQGTLVTVSSASTKGPSVFPLAPCSRSTSESTAALGCLVKDYFPEPVTVSWNSGALTSGVHTFPAVLQSSGLYSLSSVVTVPSSSLGTKTYTCNVDHKPSNTKVDKRVESKYGPPCPPCPAPEFLGGPSVFLFPPKPKDTLMISRTPEVTCVVVDVSQEDPEVQFNWYVDGVEVHNAKTKPREEQFNSTYRVVSVLTVLHQDWLNGKEYKCKVSNKGLPSSIEKTISKAKGQPREPQVYTLPPSQEEMTKNQVSLTCLVKGFYPSDIAVEWESNGQPENNYKTTPPVLDSDGSFFLYSRLTVDKSRWQEGNVFSCSVMHEALHNHYTQKSLSLSLGK

SEQ ID NO: 19 - protein, 229 aa, Artificial Sequence
  609VL-302VL(43C) amino acid sequence
EIVLTQSPATLSLSPGERATLSCRASQSISNFLHWYQQKPGQAPRLLIKYASQSISGIPARFSGSGSGTDFTLTISSLEPEDFAVYFCQQSNSWPHTFGQGTKVEIKGGGGSGGGGSGGGGSDIQMTQSPSSLSASVGDRVTITCRASQDVNTAVAWYQQKPGKCPKLLIYSASFLYSGVPSRFSGSRSGTDFTLTISSLQPEDFATYYCQQHYTTPPTFGQGTKVEIK